European Patent Application EP 4 534 657 A1, published April 9, 2025. Title: Mutant microorganism of Corynebacterium genus producing L-glutamic acid and method for producing L-glutamic acid using the same. Applicant: DAESANG CORPORATION. The sequence listing filed with the application follows.

SEQUENCE LISTING (9 sequences)

SEQ ID NO: 1 - DNA, 810 bp, synthetic construct
  source 1..810: mol_type = other DNA
atgaacgttgacatttcacgatccagagagccgctaaacgttgagctcctgaaggaaaaattgctccaaaacggtgactttggccaggtcatttacgaaaaagtgacaggctccactaatgctgacttgctggagcttgcaagctcaggcgctccaaactggacggtgaaaactgtcgagttccaagatcatgcgcgtggacgactcggccgcccgtggtctgcccctgaaggttcccaaacaatcgtgtcggtgctcgttcaactatctactgatcaattggatcgtattggcaccattccactcgcggcaggtcttgctgtcatggacgcattgaatgacctcggtgtggaaggtgccggattgaaatggcccaacgacgttcaaatccacggcaagaagctctgcggcatcctgatggaagccaccggctttgattccaccccaacagttgtcatcggttggggcactaatatcagcctgactaaagaggagcttcctgttcctcatgcaacttccctcgcattggaaggtgttgaagtcgacagaaccacattccttattaatatgctcacacatctgcatactcgactggaccagtggcagggtccaagtgtggattggctcgatgattaccgtgcggtatgttccagtattggccaagatgttcgagtgcttctacctggggataaagaactcttaggtgaagcgatcggtgtcgcgactggcggagaaattcgcgttcgcgatgcttcgggcaccgttcataccctcaacgccggtgaaattacgcaccttcgcctgcagtaa

SEQ ID NO: 2 - protein, 269 aa, synthetic construct
MNVDISRSREPLNVELLKEKLLQNGDFGQVIYEKVTGSTNADLLELASSGAPNWTVKTVEFQDHARGRLGRPWSAPEGSQTIVSVLVQLSTDQLDRIGTIPLAAGLAVMDALNDLGVEGAGLKWPNDVQIHGKKLCGILMEATGFDSTPTVVIGWGTNISLTKEELPVPHATSLALEGVEVDRTTFLINMLTHLHTRLDQWQGPSVDWLDDYRAVCSSIGQDVRVLLPGDKELLGEAIGVATGGEIRVRDASGTVHTLNAGEITHLRLQ

SEQ ID NO: 3 - DNA, 810 bp, Corynebacterium sp.
  source 1..810: mol_type = genomic DNA
atgaacgttgacatttcacgatccagagagccgctaaacgttgagctcctgaaggaaaaattgctccaaaacggtgactttggccaggtcatttacgaaaaagtgacaggctccactaatgctgacttgctggagcttgcaagctcaggcgctccaaactggacggtgaaaactgtcgagttccaagatcatgcgcgtggacgactcggccgcccgtggtctgcccctgaaggttcccaaacaatcgtgtcggtgctcgttcaactatctactgatcaattggatcgtattggcaccattccactcgcggcaggtcttgctgtcatggacgcattgaatgacctcggtgtggaaggtgccggattgaaatggcccaacgacgttcaaatccacggcaagaagctctgcggcatcctggtggaagccaccggctttgattccaccccaacagttgtcatcggttggggcactaatatcagcctgactaaagaggagcttcctgttcctcatgcaacttccctcgcattggaaggtgttgaagtcgacagaaccacattccttattaatatgctcacacatctgcatactcgactggaccagtggcagggtccaagtgtggattggctcgatgattaccgtgcggtatgttccagtattggccaagatgttcgagtgcttctacctggggataaagaactcttaggtgaagcgatcggtgtcgcgactggcggagaaattcgcgttcgcgatgcttcgggcaccgttcataccctcaacgccggtgaaattacgcaccttcgcctgcagtaa

SEQ ID NO: 4 - protein, 269 aa, Corynebacterium sp.
MNVDISRSREPLNVELLKEKLLQNGDFGQVIYEKVTGSTNADLLELASSGAPNWTVKTVEFQDHARGRLGRPWSAPEGSQTIVSVLVQLSTDQLDRIGTIPLAAGLAVMDALNDLGVEGAGLKWPNDVQIHGKKLCGILVEATGFDSTPTVVIGWGTNISLTKEELPVPHATSLALEGVEVDRTTFLINMLTHLHTRLDQWQGPSVDWLDDYRAVCSSIGQDVRVLLPGDKELLGEAIGVATGGEIRVRDASGTVHTLNAGEITHLRLQ

SEQ ID NO: 5 - DNA, 5719 bp, synthetic construct
  source 1..5719: mol_type = other DNA
tgccgcaagcactcagggcgcaagggctgctaaaggaagcggaacacgtagaaagccagtccgcagaaacggtgctgaccccggatgaatgtcagctactgggctatctggacaagggaaaacgcaagcgcaaagagaaagcaggtagcttgcagtgggcttacatggcgatagctagactgggcggttttatggacagcaagcgaaccggaattgccagctggggcgccctctggtaaggttgggaagccctgcaaagtaaactggatggctttcttgccgccaaggatctgatggcgcaggggatcaagatctgatcaagagacaggatgaggatcgtttcgcatgattgaacaagatggattgcacgcaggttctccggccgcttgggtggagaggctattcggctatgactgggcacaacagacaatcggctgctctgatgccgccgtgttccggctgtcagcgcaggggcgcccggttctttttgtcaagaccgacctgtccggtgccctgaatgaactccaagacgaggcagcgcggctatcgtggctggccacgacgggcgttccttgcgcagctgtgctcgacgttgtcactgaagcgggaagggactggctgctattgggcgaagtgccggggcaggatctcctgtcatctcaccttgctcctgccgagaaagtatccatcatggctgatgcaatgcggcggctgcatacgcttgatccggctacctgcccattcgaccaccaagcgaaacatcgcatcgagcgagcacgtactcggatggaagccggtcttgtcgatcaggatgatctggacgaagagcatcaggggctcgcgccagccgaactgttcgccaggctcaaggcgcggatgcccgacggcgaggatctcgtcgtgacccatggcgatgcctgcttgccgaatatcatggtggaaaatggccgcttttctggattcatcgactgtggccggctgggtgtggcggaccgctatcaggacatagcgttggctacccgtgatattgctgaagagcttggcggcgaatgggctgaccgcttcctcgtgctttacggtatcgccgctcccgattcgcagcgcatcgccttctatcgccttcttgacgagttcttctgagcgggactctggggttcgctagaggatcgatcctttttaacccatcacatatacctgccgttcactattatttagtgaaatgagatattatgatattttctgaattgtgattaaaaaggcaactttatgcccatgcaacagaaactataaaaaatacagagaatgaaaagaaacagatagattttttagttctttaggcccgtagtctgcaaatccttttatgattttctatcaaacaaaagaggaaaatagaccagttgcaatccaaacgagagtctaatagaatgaggtcgaaaagtaaatcgcgcgggtttgttactgataaagcaggcaagacctaaaatgtgtaaagggcaaagtgtatactttggcgtcaccccttacatattttaggtctttttttattgtgcgtaactaacttgccatcttcaaacaggagggctggaagaagcagaccgctaacacagtacataaaaaaggagacatgaacgatgaacatcaaaaagtttgcaaaacaagcaacagtattaacctttactaccgcactgctggcaggaggcgcaactcaagcgtttgcgaaagaaacgaaccaaaagccatataaggaaacatacggcatttcccatattacacgccatgatatgctgcaaatccctgaacagcaaaaaaatgaaaaatatcaagtttctgaatttgattcgtccacaattaaaaatatctcttctgcaaaaggcctggacgtttgggacagctggccattacaaaacgctgacggcactgtcgcaaactatcacggctaccacatcgtctttgcattagccggagatcctaaaaatgcggatgacacatcgatttacatgttctatcaaaaagtcggcgaaacttctattgacagctggaaaaacgctggccgcgtctttaaagacagcgacaaattcgatgcaaatgattctatcctaaaagaccaaacacaagaatggtcaggttcagccacatttacatctgacggaaaaatccgtttattctacactgatttctccggtaaacattacggcaaacaaacactgacaactgcacaagttaacgtatcagcatcagacagctctttgaacatcaacggtgtagaggattataaatcaatctttgacggtgacggaaaaacgtatcaaaatgtacagcagttcatcgatgaaggcaactacagctcaggcgacaaccatacgctgagagatcctcactacgtagaagataaaggccacaaatacttagtatttgaagcaaacactggaactgaagatggctaccaaggcgaagaatctttatttaacaaagcatactatggcaaaagcacatcattcttccgtcaagaaagtcaaaaacttctgcaaagcgataaaaaacgcacggctgagttagcaaacggcgctctcggtatgattgagctaaacgatgattacacactgaaaaaagtgatgaaaccgctgattgcatctaacacagtaacagatgaaattgaacgcgcgaacgtctttaaaatgaacggcaaatggtacctgttcactgactcccgcggatcaaaaatgacgattgacggcattacgtctaacgatatttacatgcttggttatgtttctaattctttaactggcccatacaagccgctgaacaaaactggccttgtgttaaaaatggatcttgatcctaacgatgtaacctttacttactcacacttcgctgtacctcaagcgaaaggaaacaatgtcgtgattacaagctatatgacaaacagaggattctacgcagacaaacaatcaacgtttgcgccgagcttcctgctgaacatcaaaggcaagaaaacatctgttgtcaaagacagcatccttgaacaaggacaattaacagttaacaaataaaaacgcaaaagaaaatgccgatgggtaccgagcgaaatgaccgaccaagcgacgcccaacctgccatcacgagatttcgattccaccgccgccttctatgaaaggttgggcttcggaatcgttttccgggacgccctcgcggacgtgctcatagtccacgacgcccgtgattttgtagccctggccgacggccagcaggtaggccgacaggctcatgccggccgccgccgccttttcctcaatcgctcttcgttcgtctggaaggcagtacaccttgataggtgggctgcccttcctggttggcttggtttcatcagccatccgcttgccctcatctgttacgccggcggtagccggccagcctcgcagagcaggattcccgttgagcaccgccaggtgcgaataagggacagtgaagaaggaacacccgctcgcgggtgggcctacttcacctatcctgcccggctgacgccgttggatacaccaaggaaagtctacacgaaccctttggcaaaatcctgtatatcgtgcgaaaaaggatggatataccgaaaaaatcgctataatgaccccgaagcagggttatgcagcggaaaagcgctgcttccctgctgttttgtggaatatctaccgactggaaacaggcaaatgcaggaaattactgaactgaggggacaggcgagagacgatgccaaagagctcctgaaaatctcgataactcaaaaaatacgcccggtagtgatcttatttcattatggtgaaagttggaacctcttacgtgccgatcaacgtctcattttcgccaaaagttggcccagggcttcccggtatcaacagggacaccaggatttatttattctgcgaagtgatcttccgtcacaggtatttattcggcgcaaagtgcgtcgggtgatgctgccaacttactgatttagtgtatgatggtgtttttgaggtgctccagtggcttctgtttctatcagctcctgaaaatctcgataactcaaaaaatacgcccggtagtgatcttatttcattatggtgaaagttggaacctcttacgtgccgatcaacgtctcattttcgccaaaagttggcccagggcttcccggtatcaacagggacaccaggatttatttattctgcgaagtgatcttccgtcacaggtatttattcggcgcaaagtgcgtcgggtgatgctgccaacttactgatttagtgtatgatggtgtttttgaggtgctccagtggcttctgtttctatcagggctggatgatcctccagcgcggggatctcatgctggagttcttcgcccaccccaaaaggatctaggtgaagatcctttttgataatctcatgaccaaaatcccttaacgtgagttttcgttccactgagcgtcagaccccgtagaaaagatcaaaggatcttcttgagatcctttttttctgcgcgtaatctgctgcttgcaaacaaaaaaaccaccgctaccagcggtggtttgtttgccggatcaagagctaccaactctttttccgaaggtaactggcttcagcagagcgcagataccaaatactgttcttctagtgtagccgtagttaggccaccacttcaagaactctgtagcaccgcctacatacctcgctctgctaatcctgttaccagtggctgctgccagtggcgataagtcgtgtcttaccgggttggactcaagacgatagttaccggataaggcgcagcggtcgggctgaacggggggttcgtgcacacagcccagcttggagcgaacgacctacaccgaactgagatacctacagcgtgagctatgagaaagcgccacgcttcccgaagggagaaaggcggacaggtatccggtaagcggcagggtcggaacaggagagcgcacgagggagcttccagggggaaacgcctggtatctttatagtcctgtcgggtttcgccacctctgacttgagcgtcgatttttgtgatgctcgtcaggggggcggagcctatggaaaaacgccagcaacgcggcctttttacggttcctggccttttgctggccttttgctcacatgttctttcctgcgttatcccctgattctgtggataaccgtattaccgcctttgagtgagctgataccgctcgccgcagccgaacgaccgagcgcagcgagtcagtgagcgaggaagcggaagagcgcccaatacgcaaaccgcctctccccgcgcgttggccgattcattaatgcagctggcacgacaggtttcccgactggaaagcgggcagtgagcgcaacgcaattaatgtgagttagctcactcattaggcaccccaggctttacactttatgcttccggctcgtatgttgtgtggaattgtgagcggataacaatttcacacaggaaacagctatgacatgattacgccaagcttgcatgcctgcaggtcgactctagaggatccccgggtaccgagctcgaattcactggccgtcgttttacaacgtcgtgactgggaaaaccctggcgttacccaacttaatcgccttgcagcacatccccctttcgccagctggcgtaatagcgaagaggcccgcaccgatcgcccttcccaacagttgcgcagcctgaatggcgaatggcgataagctagcttcacgc

SEQ ID NO: 6 - DNA, 20 bp, synthetic construct
  source 1..20: mol_type = other DNA
cgatgaaggagccctcatcg

SEQ ID NO: 7 - DNA, 20 bp, synthetic construct
  source 1..20: mol_type = other DNA
gtggcttccatcaggatgcc

SEQ ID NO: 8 - DNA, 20 bp, synthetic construct
  source 1..20: mol_type = other DNA
ggcatcctgatggaagccac

SEQ ID NO: 9 - DNA, 22 bp, synthetic construct
  source 1..22: mol_type = other DNA
cctaagaccagggtgtttcgcc